European Patent Specification EP 3 957 744 B1, published June 28, 2023. Title: REAGENTS AND METHODS FOR MOLECULAR BARCODING OF NUCLEIC ACIDS OF SINGLE CELLS. Applicant: CS Genetics Limited. The sequence listing filed with the application follows.

SEQUENCE LISTING (313 sequences)

SEQ ID NO: 1 - DNA, 38 bp, Artificial Sequence
  Primer
ctcgatgctacgtgactactgcgtcgaggagtctatcc

SEQ ID NO: 2 - DNA, 96 bp, Artificial Sequence
  Primer
atacctgactgctcgtcagttgagcgaattccgtatgggtagcaaggtccaagagaggctccatcctcactcgcctgactacgacaagacctactg

SEQ ID NO: 3 - DNA, 98 bp, Artificial Sequence
  Primer
tccagtaggtcttgtcgtagtcaggcgagtgaggatggagcctctcttggaccttgctacccatacggaattcgctcaactgacgagcagtcaggtat

SEQ ID NO: 4 - DNA, 22 bp, Artificial Sequence
  Primer
ctcgatgctacgtgactactgc

SEQ ID NO: 5 - DNA, 22 bp, Artificial Sequence
  Primer
cagtaggtcttgtcgtagtcag

SEQ ID NO: 6 - DNA, 45 bp, Artificial Sequence
  Primer
atggtacacacctacactactcggacgctcttccgatcttgacct

SEQ ID NO: 7 - DNA, 44 bp, Artificial Sequence
  Primer
aggtcaagatcggaagagcgtccgagtagtgtaggtgtgtacca

SEQ ID NO: 8 - DNA, 22 bp, Artificial Sequence
  Primer
tggtacacacctacactactcg

SEQ ID NO: 9 - DNA, 20 bp, Artificial Sequence
  Primer
ccatacggaattcgctcaac

SEQ ID NO: 10 - DNA, 42 bp, Artificial Sequence
  Primer
gttgagcgaattccgtatggtggtacacacctacactactcg

SEQ ID NO: 11 - DNA, 46 bp, Artificial Sequence
  Primer
taggacgatacgagtgtgtactcgtggtacacacctacactactcg

SEQ ID NO: 12 - DNA, 42 bp, Artificial Sequence
  Primer
cgagtagtgtaggtgtgtaccaccatacggaattcgctcaac

SEQ ID NO: 13 - DNA, 44 bp, Artificial Sequence
  Primer
ctgtcaaggtagactagcatgctcccatacggaattcgctcaac

SEQ ID NO: 14 - DNA, 24 bp, Artificial Sequence
  Primer
taggacgatacgagtgtgtactcg

SEQ ID NO: 15 - DNA, 24 bp, Artificial Sequence
  Primer
ctgtcaaggtagactagcatgctc

SEQ ID NO: 16 - DNA, 56 bp, Artificial Sequence
  Primer
ctcggcattcctgctgaaccgctcttccgatctgctcaactgacgagcagtcaggt

SEQ ID NO: 17 - DNA, 39 bp, Artificial Sequence
  Primer
acactctttccctacacgacgctcttccgatcttgacct

SEQ ID NO: 18 - DNA, 20 bp, Artificial Sequence
  Sequence used in the synthesis of sub-barcode molecule library
aaacggatagactcctcgac

SEQ ID NO: 19 - DNA, 20 bp, Artificial Sequence
  Sequence used in the synthesis of sub-barcode molecule library
aaagggatagactcctcgac

SEQ ID NO: 20 - DNA, 20 bp, Artificial Sequence
  Sequence used in the synthesis of sub-barcode molecule library
aaatggatagactcctcgac

SEQ ID NO: 21 - DNA, 20 bp, Artificial Sequence
  Sequence used in the synthesis of sub-barcode molecule library
aacaggatagactcctcgac

SEQ ID NO: 22 - DNA, 20 bp, Artificial Sequence
  Sequence used in the synthesis of sub-barcode molecule library
aaccggatagactcctcgac

SEQ ID NO: 23 - DNA, 20 bp, Artificial Sequence
  Sequence used in the synthesis of sub-barcode molecule library
aacgggatagactcctcgac

SEQ ID NO: 24 - DNA, 20 bp, Artificial Sequence
  Sequence used in the synthesis of sub-barcode molecule library
aactggatagactcctcgac

SEQ ID NO: 25 - DNA, 20 bp, Artificial Sequence
  Sequence used in the synthesis of sub-barcode molecule library
aagaggatagactcctcgac

SEQ ID NO: 26 - DNA, 20 bp, Artificial Sequence
  Sequence used in the synthesis of sub-barcode molecule library
aagcggatagactcctcgac

SEQ ID NO: 27 - DNA, 20 bp, Artificial Sequence
  Sequence used in the synthesis of sub-barcode molecule library
aaggggatagactcctcgac

SEQ ID NO: 28 - DNA, 20 bp, Artificial Sequence
  Sequence used in the synthesis of sub-barcode molecule library
aagtggatagactcctcgac

SEQ ID NO: 29 - DNA, 20 bp, Artificial Sequence
  Sequence used in the synthesis of sub-barcode molecule library
aataggatagactcctcgac

SEQ ID NO: 30 - DNA, 20 bp, Artificial Sequence
  Sequence used in the synthesis of sub-barcode molecule library
aatcggatagactcctcgac

SEQ ID NO: 31 - DNA, 20 bp, Artificial Sequence
  Sequence used in the synthesis of sub-barcode molecule library
aatgggatagactcctcgac

SEQ ID NO: 32 - DNA, 20 bp, Artificial Sequence
  Sequence used in the synthesis of sub-barcode molecule library
aattggatagactcctcgac

SEQ ID NO: 33 - DNA, 20 bp, Artificial Sequence
  Sequence used in the synthesis of sub-barcode molecule library
acaaggatagactcctcgac

SEQ ID NO: 34 - DNA, 20 bp, Artificial Sequence
  Sequence used in the synthesis of sub-barcode molecule library
acacggatagactcctcgac

SEQ ID NO: 35 - DNA, 20 bp, Artificial Sequence
  Sequence used in the synthesis of sub-barcode molecule library
acagggatagactcctcgac

SEQ ID NO: 36 - DNA, 20 bp, Artificial Sequence
  Sequence used in the synthesis of sub-barcode molecule library
acatggatagactcctcgac

SEQ ID NO: 37 - DNA, 20 bp, Artificial Sequence
  Sequence used in the synthesis of sub-barcode molecule library
accaggatagactcctcgac

SEQ ID NO: 38 - DNA, 20 bp, Artificial Sequence
  Sequence used in the synthesis of sub-barcode molecule library
acccggatagactcctcgac

SEQ ID NO: 39 - DNA, 20 bp, Artificial Sequence
  Sequence used in the synthesis of sub-barcode molecule library
accgggatagactcctcgac

SEQ ID NO: 40 - DNA, 20 bp, Artificial Sequence
  Sequence used in the synthesis of sub-barcode molecule library
acctggatagactcctcgac

SEQ ID NO: 41 - DNA, 20 bp, Artificial Sequence
  Sequence used in the synthesis of sub-barcode molecule library
acgaggatagactcctcgac

SEQ ID NO: 42 - DNA, 20 bp, Artificial Sequence
  Sequence used in the synthesis of sub-barcode molecule library
acgcggatagactcctcgac

SEQ ID NO: 43 - DNA, 20 bp, Artificial Sequence
  Sequence used in the synthesis of sub-barcode molecule library
acggggatagactcctcgac

SEQ ID NO: 44 - DNA, 20 bp, Artificial Sequence
  Sequence used in the synthesis of sub-barcode molecule library
acgtggatagactcctcgac

SEQ ID NO: 45 - DNA, 20 bp, Artificial Sequence
  Sequence used in the synthesis of sub-barcode molecule library
actaggatagactcctcgac

SEQ ID NO: 46 - DNA, 20 bp, Artificial Sequence
  Sequence used in the synthesis of sub-barcode molecule library
actcggatagactcctcgac

SEQ ID NO: 47 - DNA, 20 bp, Artificial Sequence
  Sequence used in the synthesis of sub-barcode molecule library
actgggatagactcctcgac

SEQ ID NO: 48 - DNA, 20 bp, Artificial Sequence
  Sequence used in the synthesis of sub-barcode molecule library
acttggatagactcctcgac

SEQ ID NO: 49 - DNA, 20 bp, Artificial Sequence
  Sequence used in the synthesis of sub-barcode molecule library
agaaggatagactcctcgac

SEQ ID NO: 50 - DNA, 20 bp, Artificial Sequence
  Sequence used in the synthesis of sub-barcode molecule library
agacggatagactcctcgac

SEQ ID NO: 51 - DNA, 20 bp, Artificial Sequence
  Sequence used in the synthesis of sub-barcode molecule library
agagggatagactcctcgac

SEQ ID NO: 52 - DNA, 20 bp, Artificial Sequence
  Sequence used in the synthesis of sub-barcode molecule library
agatggatagactcctcgac

SEQ ID NO: 53 - DNA, 20 bp, Artificial Sequence
  Sequence used in the synthesis of sub-barcode molecule library
agcaggatagactcctcgac

SEQ ID NO: 54 - DNA, 20 bp, Artificial Sequence
  Sequence used in the synthesis of sub-barcode molecule library
agccggatagactcctcgac

SEQ ID NO: 55 - DNA, 20 bp, Artificial Sequence
  Sequence used in the synthesis of sub-barcode molecule library
agcgggatagactcctcgac

SEQ ID NO: 56 - DNA, 20 bp, Artificial Sequence
  Sequence used in the synthesis of sub-barcode molecule library
agctggatagactcctcgac

SEQ ID NO: 57 - DNA, 20 bp, Artificial Sequence
  Sequence used in the synthesis of sub-barcode molecule library
aggaggatagactcctcgac

SEQ ID NO: 58 - DNA, 20 bp, Artificial Sequence
  Sequence used in the synthesis of sub-barcode molecule library
aggcggatagactcctcgac

SEQ ID NO: 59 - DNA, 20 bp, Artificial Sequence
  Sequence used in the synthesis of sub-barcode molecule library
agggggatagactcctcgac

SEQ ID NO: 60 - DNA, 20 bp, Artificial Sequence
  Sequence used in the synthesis of sub-barcode molecule library
aggtggatagactcctcgac

SEQ ID NO: 61 - DNA, 20 bp, Artificial Sequence
  Sequence used in the synthesis of sub-barcode molecule library
agtaggatagactcctcgac

SEQ ID NO: 62 - DNA, 20 bp, Artificial Sequence
  Sequence used in the synthesis of sub-barcode molecule library
agtcggatagactcctcgac

SEQ ID NO: 63 - DNA, 20 bp, Artificial Sequence
  Sequence used in the synthesis of sub-barcode molecule library
agtgggatagactcctcgac

SEQ ID NO: 64 - DNA, 20 bp, Artificial Sequence
  Sequence used in the synthesis of sub-barcode molecule library
agttggatagactcctcgac

SEQ ID NO: 65 - DNA, 20 bp, Artificial Sequence
  Sequence used in the synthesis of sub-barcode molecule library
ataaggatagactcctcgac

SEQ ID NO: 66 - DNA, 20 bp, Artificial Sequence
  Sequence used in the synthesis of sub-barcode molecule library
atacggatagactcctcgac

SEQ ID NO: 67 - DNA, 20 bp, Artificial Sequence
  Sequence used in the synthesis of sub-barcode molecule library
atagggatagactcctcgac

SEQ ID NO: 68 - DNA, 20 bp, Artificial Sequence
  Sequence used in the synthesis of sub-barcode molecule library
atatggatagactcctcgac

SEQ ID NO: 69 - DNA, 20 bp, Artificial Sequence
  Sequence used in the synthesis of sub-barcode molecule library
atcaggatagactcctcgac

SEQ ID NO: 70 - DNA, 20 bp, Artificial Sequence
  Sequence used in the synthesis of sub-barcode molecule library
atccggatagactcctcgac

SEQ ID NO: 71 - DNA, 20 bp, Artificial Sequence
  Sequence used in the synthesis of sub-barcode molecule library
atcgggatagactcctcgac

SEQ ID NO: 72 - DNA, 20 bp, Artificial Sequence
  Sequence used in the synthesis of sub-barcode molecule library
atctggatagactcctcgac

SEQ ID NO: 73 - DNA, 20 bp, Artificial Sequence
  Sequence used in the synthesis of sub-barcode molecule library
atgaggatagactcctcgac

SEQ ID NO: 74 - DNA, 20 bp, Artificial Sequence
  Sequence used in the synthesis of sub-barcode molecule library
atgcggatagactcctcgac

SEQ ID NO: 75 - DNA, 20 bp, Artificial Sequence
  Sequence used in the synthesis of sub-barcode molecule library
atggggatagactcctcgac

SEQ ID NO: 76 - DNA, 20 bp, Artificial Sequence
  Sequence used in the synthesis of sub-barcode molecule library
atgtggatagactcctcgac

SEQ ID NO: 77 - DNA, 20 bp, Artificial Sequence
  Sequence used in the synthesis of sub-barcode molecule library
attaggatagactcctcgac

SEQ ID NO: 78 - DNA, 20 bp, Artificial Sequence
  Sequence used in the synthesis of sub-barcode molecule library
attcggatagactcctcgac

SEQ ID NO: 79 - DNA, 20 bp, Artificial Sequence
  Sequence used in the synthesis of sub-barcode molecule library
attgggatagactcctcgac

SEQ ID NO: 80 - DNA, 20 bp, Artificial Sequence
  Sequence used in the synthesis of sub-barcode molecule library
atttggatagactcctcgac

SEQ ID NO: 81 - DNA, 20 bp, Artificial Sequence
  Sequence used in the synthesis of sub-barcode molecule library
caaaggatagactcctcgac

SEQ ID NO: 82 - DNA, 20 bp, Artificial Sequence
  Sequence used in the synthesis of sub-barcode molecule library
caacggatagactcctcgac

SEQ ID NO: 83 - DNA, 20 bp, Artificial Sequence
  Sequence used in the synthesis of sub-barcode molecule library
caagggatagactcctcgac

SEQ ID NO: 84 - DNA, 20 bp, Artificial Sequence
  Sequence used in the synthesis of sub-barcode molecule library
caatggatagactcctcgac

SEQ ID NO: 85 - DNA, 20 bp, Artificial Sequence
  Sequence used in the synthesis of sub-barcode molecule library
cacaggatagactcctcgac

SEQ ID NO: 86 - DNA, 20 bp, Artificial Sequence
  Sequence used in the synthesis of sub-barcode molecule library
caccggatagactcctcgac

SEQ ID NO: 87 - DNA, 20 bp, Artificial Sequence
  Sequence used in the synthesis of sub-barcode molecule library
cacgggatagactcctcgac

SEQ ID NO: 88 - DNA, 20 bp, Artificial Sequence
  Sequence used in the synthesis of sub-barcode molecule library
cactggatagactcctcgac

SEQ ID NO: 89 - DNA, 20 bp, Artificial Sequence
  Sequence used in the synthesis of sub-barcode molecule library
cagaggatagactcctcgac

SEQ ID NO: 90 - DNA, 20 bp, Artificial Sequence
  Sequence used in the synthesis of sub-barcode molecule library
cagcggatagactcctcgac

SEQ ID NO: 91 - DNA, 20 bp, Artificial Sequence
  Sequence used in the synthesis of sub-barcode molecule library
caggggatagactcctcgac

SEQ ID NO: 92 - DNA, 20 bp, Artificial Sequence
  Sequence used in the synthesis of sub-barcode molecule library
cagtggatagactcctcgac

SEQ ID NO: 93 - DNA, 20 bp, Artificial Sequence
  Sequence used in the synthesis of sub-barcode molecule library
cataggatagactcctcgac

SEQ ID NO: 94 - DNA, 20 bp, Artificial Sequence
  Sequence used in the synthesis of sub-barcode molecule library
catcggatagactcctcgac

SEQ ID NO: 95 - DNA, 20 bp, Artificial Sequence
  Sequence used in the synthesis of sub-barcode molecule library
catgggatagactcctcgac

SEQ ID NO: 96 - DNA, 20 bp, Artificial Sequence
  Sequence used in the synthesis of sub-barcode molecule library
cattggatagactcctcgac

SEQ ID NO: 97 - DNA, 20 bp, Artificial Sequence
  Sequence used in the synthesis of sub-barcode molecule library
ccaaggatagactcctcgac

SEQ ID NO: 98 - DNA, 20 bp, Artificial Sequence
  Sequence used in the synthesis of sub-barcode molecule library
ccacggatagactcctcgac

SEQ ID NO: 99 - DNA, 20 bp, Artificial Sequence
  Sequence used in the synthesis of sub-barcode molecule library
ccagggatagactcctcgac

SEQ ID NO: 100 - DNA, 20 bp, Artificial Sequence
  Sequence used in the synthesis of sub-barcode molecule library
ccatggatagactcctcgac

SEQ ID NO: 101 - DNA, 20 bp, Artificial Sequence
  Sequence used in the synthesis of sub-barcode molecule library
cccaggatagactcctcgac

SEQ ID NO: 102 - DNA, 20 bp, Artificial Sequence
  Sequence used in the synthesis of sub-barcode molecule library
cccgggatagactcctcgac

SEQ ID NO: 103 - DNA, 20 bp, Artificial Sequence
  Sequence used in the synthesis of sub-barcode molecule library
ccctggatagactcctcgac

SEQ ID NO: 104 - DNA, 20 bp, Artificial Sequence
  Sequence used in the synthesis of sub-barcode molecule library
ccgaggatagactcctcgac

SEQ ID NO: 105 - DNA, 20 bp, Artificial Sequence
  Sequence used in the synthesis of sub-barcode molecule library
ccgcggatagactcctcgac

SEQ ID NO: 106 - DNA, 20 bp, Artificial Sequence
  Sequence used in the synthesis of sub-barcode molecule library
ccggggatagactcctcgac

SEQ ID NO: 107 - DNA, 20 bp, Artificial Sequence
  Sequence used in the synthesis of sub-barcode molecule library
ccgtggatagactcctcgac

SEQ ID NO: 108 - DNA, 20 bp, Artificial Sequence
  Sequence used in the synthesis of sub-barcode molecule library
cctaggatagactcctcgac

SEQ ID NO: 109 - DNA, 20 bp, Artificial Sequence
  Sequence used in the synthesis of sub-barcode molecule library
cctcggatagactcctcgac

SEQ ID NO: 110 - DNA, 20 bp, Artificial Sequence
  Sequence used in the synthesis of sub-barcode molecule library
cctgggatagactcctcgac

SEQ ID NO: 111 - DNA, 20 bp, Artificial Sequence
  Sequence used in the synthesis of sub-barcode molecule library
ccttggatagactcctcgac

SEQ ID NO: 112 - DNA, 20 bp, Artificial Sequence
  Sequence used in the synthesis of sub-barcode molecule library
cgaaggatagactcctcgac

SEQ ID NO: 113 - DNA, 20 bp, Artificial Sequence
  Sequence used in the synthesis of sub-barcode molecule library
cgacggatagactcctcgac

SEQ ID NO: 114 - DNA, 20 bp, Artificial Sequence
  Sequence used in the synthesis of sub-barcode molecule library
cgagggatagactcctcgac

SEQ ID NO: 115 - DNA, 20 bp, Artificial Sequence
  Sequence used in the synthesis of sub-barcode molecule library
cgatggatagactcctcgac

SEQ ID NO: 116 - DNA, 20 bp, Artificial Sequence
  Sequence used in the synthesis of sub-barcode molecule library
cgcaggatagactcctcgac

SEQ ID NO: 117 - DNA, 20 bp, Artificial Sequence
  Sequence used in the synthesis of sub-barcode molecule library
cgccggatagactcctcgac

SEQ ID NO: 118 - DNA, 20 bp, Artificial Sequence
  Sequence used in the synthesis of sub-barcode molecule library
cgcgggatagactcctcgac

SEQ ID NO: 119 - DNA, 20 bp, Artificial Sequence
  Sequence used in the synthesis of sub-barcode molecule library
cgctggatagactcctcgac

SEQ ID NO: 120 - DNA, 20 bp, Artificial Sequence
  Sequence used in the synthesis of sub-barcode molecule library
cggaggatagactcctcgac

SEQ ID NO: 121 - DNA, 20 bp, Artificial Sequence
  Sequence used in the synthesis of sub-barcode molecule library
cggcggatagactcctcgac

SEQ ID NO: 122 - DNA, 20 bp, Artificial Sequence
  Sequence used in the synthesis of sub-barcode molecule library
cgggggatagactcctcgac

SEQ ID NO: 123 - DNA, 20 bp, Artificial Sequence
  Sequence used in the synthesis of sub-barcode molecule library
cggtggatagactcctcgac

SEQ ID NO: 124 - DNA, 20 bp, Artificial Sequence
  Sequence used in the synthesis of sub-barcode molecule library
cgtaggatagactcctcgac

SEQ ID NO: 125 - DNA, 20 bp, Artificial Sequence
  Sequence used in the synthesis of sub-barcode molecule library
cgtcggatagactcctcgac

SEQ ID NO: 126 - DNA, 20 bp, Artificial Sequence
  Sequence used in the synthesis of sub-barcode molecule library
cgtgggatagactcctcgac

SEQ ID NO: 127 - DNA, 20 bp, Artificial Sequence
  Sequence used in the synthesis of sub-barcode molecule library
cgttggatagactcctcgac

SEQ ID NO: 128 - DNA, 20 bp, Artificial Sequence
  Sequence used in the synthesis of sub-barcode molecule library
ctaaggatagactcctcgac

SEQ ID NO: 129 - DNA, 20 bp, Artificial Sequence
  Sequence used in the synthesis of sub-barcode molecule library
ctacggatagactcctcgac

SEQ ID NO: 130 - DNA, 20 bp, Artificial Sequence
  Sequence used in the synthesis of sub-barcode molecule library
ctagggatagactcctcgac

SEQ ID NO: 131 - DNA, 20 bp, Artificial Sequence
  Sequence used in the synthesis of sub-barcode molecule library
ctatggatagactcctcgac

SEQ ID NO: 132 - DNA, 20 bp, Artificial Sequence
  Sequence used in the synthesis of sub-barcode molecule library
ctcaggatagactcctcgac

SEQ ID NO: 133 - DNA, 20 bp, Artificial Sequence
  Sequence used in the synthesis of sub-barcode molecule library
ctccggatagactcctcgac

SEQ ID NO: 134 - DNA, 20 bp, Artificial Sequence
  Sequence used in the synthesis of sub-barcode molecule library
ctcgggatagactcctcgac

SEQ ID NO: 135 - DNA, 20 bp, Artificial Sequence
  Sequence used in the synthesis of sub-barcode molecule library
ctctggatagactcctcgac

SEQ ID NO: 136 - DNA, 20 bp, Artificial Sequence
  Sequence used in the synthesis of sub-barcode molecule library
ctgaggatagactcctcgac

SEQ ID NO: 137 - DNA, 20 bp, Artificial Sequence
  Sequence used in the synthesis of sub-barcode molecule library
ctgcggatagactcctcgac

SEQ ID NO: 138 - DNA, 20 bp, Artificial Sequence
  Sequence used in the synthesis of sub-barcode molecule library
ctggggatagactcctcgac

SEQ ID NO: 139 - DNA, 20 bp, Artificial Sequence
  Sequence used in the synthesis of sub-barcode molecule library
ctgtggatagactcctcgac

SEQ ID NO: 140 - DNA, 20 bp, Artificial Sequence
  Sequence used in the synthesis of sub-barcode molecule library
cttaggatagactcctcgac

SEQ ID NO: 141 - DNA, 20 bp, Artificial Sequence
  Sequence used in the synthesis of sub-barcode molecule library
cttcggatagactcctcgac

SEQ ID NO: 142 - DNA, 20 bp, Artificial Sequence
  Sequence used in the synthesis of sub-barcode molecule library
cttgggatagactcctcgac

SEQ ID NO: 143 - DNA, 20 bp, Artificial Sequence
  Sequence used in the synthesis of sub-barcode molecule library
ctttggatagactcctcgac

SEQ ID NO: 144 - DNA, 20 bp, Artificial Sequence
  Sequence used in the synthesis of sub-barcode molecule library
gaaaggatagactcctcgac

SEQ ID NO: 145 - DNA, 20 bp, Artificial Sequence
  Sequence used in the synthesis of sub-barcode molecule library
gaacggatagactcctcgac

SEQ ID NO: 146 - DNA, 20 bp, Artificial Sequence
  Sequence used in the synthesis of sub-barcode molecule library
gaagggatagactcctcgac

SEQ ID NO: 147 - DNA, 20 bp, Artificial Sequence
  Sequence used in the synthesis of sub-barcode molecule library
gaatggatagactcctcgac

SEQ ID NO: 148 - DNA, 20 bp, Artificial Sequence
  Sequence used in the synthesis of sub-barcode molecule library
gacaggatagactcctcgac

SEQ ID NO: 149 - DNA, 20 bp, Artificial Sequence
  Sequence used in the synthesis of sub-barcode molecule library
gaccggatagactcctcgac

SEQ ID NO: 150 - DNA, 20 bp, Artificial Sequence
  Sequence used in the synthesis of sub-barcode molecule library
gacgggatagactcctcgac

SEQ ID NO: 151 - DNA, 20 bp, Artificial Sequence
  Sequence used in the synthesis of sub-barcode molecule library
gactggatagactcctcgac

SEQ ID NO: 152 - DNA, 20 bp, Artificial Sequence
  Sequence used in the synthesis of sub-barcode molecule library
gagaggatagactcctcgac

SEQ ID NO: 153 - DNA, 20 bp, Artificial Sequence
  Sequence used in the synthesis of sub-barcode molecule library
gagcggatagactcctcgac

SEQ ID NO: 154 - DNA, 20 bp, Artificial Sequence
  Sequence used in the synthesis of sub-barcode molecule library
gaggggatagactcctcgac

SEQ ID NO: 155 - DNA, 20 bp, Artificial Sequence
  Sequence used in the synthesis of sub-barcode molecule library
gagtggatagactcctcgac

SEQ ID NO: 156 - DNA, 20 bp, Artificial Sequence
  Sequence used in the synthesis of sub-barcode molecule library
gataggatagactcctcgac

SEQ ID NO: 157 - DNA, 20 bp, Artificial Sequence
  Sequence used in the synthesis of sub-barcode molecule library
gatcggatagactcctcgac

SEQ ID NO: 158 - DNA, 20 bp, Artificial Sequence
  Sequence used in the synthesis of sub-barcode molecule library
gatgggatagactcctcgac

SEQ ID NO: 159 - DNA, 20 bp, Artificial Sequence
  Sequence used in the synthesis of sub-barcode molecule library
gattggatagactcctcgac

SEQ ID NO: 160 - DNA, 20 bp, Artificial Sequence
  Sequence used in the synthesis of sub-barcode molecule library
gcaaggatagactcctcgac

SEQ ID NO: 161 - DNA, 20 bp, Artificial Sequence
  Sequence used in the synthesis of sub-barcode molecule library
gcacggatagactcctcgac

SEQ ID NO: 162 - DNA, 20 bp, Artificial Sequence
  Sequence used in the synthesis of sub-barcode molecule library
gcagggatagactcctcgac

SEQ ID NO: 163 - DNA, 20 bp, Artificial Sequence
  Sequence used in the synthesis of sub-barcode molecule library
gcatggatagactcctcgac

SEQ ID NO: 164 - DNA, 20 bp, Artificial Sequence
  Sequence used in the synthesis of sub-barcode molecule library
gccaggatagactcctcgac

SEQ ID NO: 165 - DNA, 20 bp, Artificial Sequence
  Sequence used in the synthesis of sub-barcode molecule library
gcccggatagactcctcgac

SEQ ID NO: 166 - DNA, 20 bp, Artificial Sequence
  Sequence used in the synthesis of sub-barcode molecule library
gccgggatagactcctcgac

SEQ ID NO: 167 - DNA, 20 bp, Artificial Sequence
  Sequence used in the synthesis of sub-barcode molecule library
gcctggatagactcctcgac

SEQ ID NO: 168 - DNA, 20 bp, Artificial Sequence
  Sequence used in the synthesis of sub-barcode molecule library
gcgaggatagactcctcgac

SEQ ID NO: 169 - DNA, 20 bp, Artificial Sequence
  Sequence used in the synthesis of sub-barcode molecule library
gcgcggatagactcctcgac

SEQ ID NO: 170 - DNA, 20 bp, Artificial Sequence
  Sequence used in the synthesis of sub-barcode molecule library
gcggggatagactcctcgac

SEQ ID NO: 171 - DNA, 20 bp, Artificial Sequence
  Sequence used in the synthesis of sub-barcode molecule library
gcgtggatagactcctcgac

SEQ ID NO: 172 - DNA, 20 bp, Artificial Sequence
  Sequence used in the synthesis of sub-barcode molecule library
gctaggatagactcctcgac

SEQ ID NO: 173 - DNA, 20 bp, Artificial Sequence
  Sequence used in the synthesis of sub-barcode molecule library
gctcggatagactcctcgac

SEQ ID NO: 174 - DNA, 20 bp, Artificial Sequence
  Sequence used in the synthesis of sub-barcode molecule library
gctgggatagactcctcgac

SEQ ID NO: 175 - DNA, 20 bp, Artificial Sequence
  Sequence used in the synthesis of sub-barcode molecule library
gcttggatagactcctcgac

SEQ ID NO: 176 - DNA, 20 bp, Artificial Sequence
  Sequence used in the synthesis of sub-barcode molecule library
ggaaggatagactcctcgac

SEQ ID NO: 177 - DNA, 20 bp, Artificial Sequence
  Sequence used in the synthesis of sub-barcode molecule library
ggacggatagactcctcgac

SEQ ID NO: 178 - DNA, 20 bp, Artificial Sequence
  Sequence used in the synthesis of sub-barcode molecule library
ggagggatagactcctcgac

SEQ ID NO: 179 - DNA, 20 bp, Artificial Sequence
  Sequence used in the synthesis of sub-barcode molecule library
ggatggatagactcctcgac

SEQ ID NO: 180 - DNA, 20 bp, Artificial Sequence
  Sequence used in the synthesis of sub-barcode molecule library
ggcaggatagactcctcgac

SEQ ID NO: 181 - DNA, 20 bp, Artificial Sequence
  Sequence used in the synthesis of sub-barcode molecule library
ggccggatagactcctcgac

SEQ ID NO: 182 - DNA, 20 bp, Artificial Sequence
  Sequence used in the synthesis of sub-barcode molecule library
ggcgggatagactcctcgac

SEQ ID NO: 183 - DNA, 20 bp, Artificial Sequence
  Sequence used in the synthesis of sub-barcode molecule library
ggctggatagactcctcgac

SEQ ID NO: 184 - DNA, 20 bp, Artificial Sequence
  Sequence used in the synthesis of sub-barcode molecule library
gggaggatagactcctcgac

SEQ ID NO: 185 - DNA, 20 bp, Artificial Sequence
  Sequence used in the synthesis of sub-barcode molecule library
gggcggatagactcctcgac

SEQ ID NO: 186 - DNA, 20 bp, Artificial Sequence
  Sequence used in the synthesis of sub-barcode molecule library
gggtggatagactcctcgac

SEQ ID NO: 187 - DNA, 20 bp, Artificial Sequence
  Sequence used in the synthesis of sub-barcode molecule library
ggtaggatagactcctcgac

SEQ ID NO: 188 - DNA, 20 bp, Artificial Sequence
  Sequence used in the synthesis of sub-barcode molecule library
ggtcggatagactcctcgac

SEQ ID NO: 189 - DNA, 20 bp, Artificial Sequence
  Sequence used in the synthesis of sub-barcode molecule library
ggtgggatagactcctcgac

SEQ ID NO: 190 - DNA, 20 bp, Artificial Sequence
  Sequence used in the synthesis of sub-barcode molecule library
ggttggatagactcctcgac

SEQ ID NO: 191 - DNA, 20 bp, Artificial Sequence
  Sequence used in the synthesis of sub-barcode molecule library
gtaaggatagactcctcgac

SEQ ID NO: 192 - DNA, 20 bp, Artificial Sequence
  Sequence used in the synthesis of sub-barcode molecule library
gtacggatagactcctcgac

SEQ ID NO: 193 - DNA, 20 bp, Artificial Sequence
  Sequence used in the synthesis of sub-barcode molecule library
gtagggatagactcctcgac

SEQ ID NO: 194 - DNA, 20 bp, Artificial Sequence
  Sequence used in the synthesis of sub-barcode molecule library
gtatggatagactcctcgac

SEQ ID NO: 195 - DNA, 20 bp, Artificial Sequence
  Sequence used in the synthesis of sub-barcode molecule library
gtcaggatagactcctcgac

SEQ ID NO: 196 - DNA, 20 bp, Artificial Sequence
  Sequence used in the synthesis of sub-barcode molecule library
gtccggatagactcctcgac

SEQ ID NO: 197 - DNA, 20 bp, Artificial Sequence
  Sequence used in the synthesis of sub-barcode molecule library
gtcgggatagactcctcgac

SEQ ID NO: 198 - DNA, 20 bp, Artificial Sequence
  Sequence used in the synthesis of sub-barcode molecule library
gtctggatagactcctcgac

SEQ ID NO: 199 - DNA, 20 bp, Artificial Sequence
  Sequence used in the synthesis of sub-barcode molecule library
gtgaggatagactcctcgac

SEQ ID NO: 200 - DNA, 20 bp, Artificial Sequence
  Sequence used in the synthesis of sub-barcode molecule library
gtgcggatagactcctcgac

SEQ ID NO: 201 - DNA, 20 bp, Artificial Sequence
  Sequence used in the synthesis of sub-barcode molecule library
gtggggatagactcctcgac

SEQ ID NO: 202 - DNA, 20 bp, Artificial Sequence
  Sequence used in the synthesis of sub-barcode molecule library
gtgtggatagactcctcgac

SEQ ID NO: 203 - DNA, 20 bp, Artificial Sequence
  Sequence used in the synthesis of sub-barcode molecule library
gttaggatagactcctcgac

SEQ ID NO: 204 - DNA, 20 bp, Artificial Sequence
  Sequence used in the synthesis of sub-barcode molecule library
gttcggatagactcctcgac

SEQ ID NO: 205 - DNA, 20 bp, Artificial Sequence
  Sequence used in the synthesis of sub-barcode molecule library
gttgggatagactcctcgac

SEQ ID NO: 206 - DNA, 20 bp, Artificial Sequence
  Sequence used in the synthesis of sub-barcode molecule library
gtttggatagactcctcgac

SEQ ID NO: 207 - DNA, 20 bp, Artificial Sequence
  Sequence used in the synthesis of sub-barcode molecule library
taaaggatagactcctcgac

SEQ ID NO: 208 - DNA, 20 bp, Artificial Sequence
  Sequence used in the synthesis of sub-barcode molecule library
taacggatagactcctcgac

SEQ ID NO: 209 - DNA, 20 bp, Artificial Sequence
  Sequence used in the synthesis of sub-barcode molecule library
taagggatagactcctcgac

SEQ ID NO: 210 - DNA, 20 bp, Artificial Sequence
  Sequence used in the synthesis of sub-barcode molecule library
taatggatagactcctcgac

SEQ ID NO: 211 - DNA, 20 bp, Artificial Sequence
  Sequence used in the synthesis of sub-barcode molecule library
tacaggatagactcctcgac

SEQ ID NO: 212 - DNA, 20 bp, Artificial Sequence
  Sequence used in the synthesis of sub-barcode molecule library
taccggatagactcctcgac

SEQ ID NO: 213 - DNA, 20 bp, Artificial Sequence
  Sequence used in the synthesis of sub-barcode molecule library
tacgggatagactcctcgac

SEQ ID NO: 214 - DNA, 20 bp, Artificial Sequence
  Sequence used in the synthesis of sub-barcode molecule library
tactggatagactcctcgac

SEQ ID NO: 215 - DNA, 20 bp, Artificial Sequence
  Sequence used in the synthesis of sub-barcode molecule library
tagaggatagactcctcgac

SEQ ID NO: 216 - DNA, 20 bp, Artificial Sequence
  Sequence used in the synthesis of sub-barcode molecule library
tagcggatagactcctcgac

SEQ ID NO: 217 - DNA, 20 bp, Artificial Sequence
  Sequence used in the synthesis of sub-barcode molecule library
taggggatagactcctcgac

SEQ ID NO: 218 - DNA, 20 bp, Artificial Sequence
  Sequence used in the synthesis of sub-barcode molecule library
tagtggatagactcctcgac

SEQ ID NO: 219 - DNA, 20 bp, Artificial Sequence
  Sequence used in the synthesis of sub-barcode molecule library
tataggatagactcctcgac

SEQ ID NO: 220 - DNA, 20 bp, Artificial Sequence
  Sequence used in the synthesis of sub-barcode molecule library
tatcggatagactcctcgac

SEQ ID NO: 221 - DNA, 20 bp, Artificial Sequence
  Sequence used in the synthesis of sub-barcode molecule library
tatgggatagactcctcgac

SEQ ID NO: 222 - DNA, 20 bp, Artificial Sequence
  Sequence used in the synthesis of sub-barcode molecule library
tattggatagactcctcgac

SEQ ID NO: 223 - DNA, 20 bp, Artificial Sequence
  Sequence used in the synthesis of sub-barcode molecule library
tcaaggatagactcctcgac

SEQ ID NO: 224 - DNA, 20 bp, Artificial Sequence
  Sequence used in the synthesis of sub-barcode molecule library
tcacggatagactcctcgac

SEQ ID NO: 225 - DNA, 20 bp, Artificial Sequence
  Sequence used in the synthesis of sub-barcode molecule library
tcagggatagactcctcgac

SEQ ID NO: 226 - DNA, 20 bp, Artificial Sequence
  Sequence used in the synthesis of sub-barcode molecule library
tcatggatagactcctcgac

SEQ ID NO: 227 - DNA, 20 bp, Artificial Sequence
  Sequence used in the synthesis of sub-barcode molecule library
tccaggatagactcctcgac

SEQ ID NO: 228 - DNA, 20 bp, Artificial Sequence
  Sequence used in the synthesis of sub-barcode molecule library
tcccggatagactcctcgac

SEQ ID NO: 229 - DNA, 20 bp, Artificial Sequence
  Sequence used in the synthesis of sub-barcode molecule library
tccgggatagactcctcgac

SEQ ID NO: 230 - DNA, 20 bp, Artificial Sequence
  Sequence used in the synthesis of sub-barcode molecule library
tcctggatagactcctcgac

SEQ ID NO: 231 - DNA, 20 bp, Artificial Sequence
  Sequence used in the synthesis of sub-barcode molecule library
tcgaggatagactcctcgac

SEQ ID NO: 232 - DNA, 20 bp, Artificial Sequence
  Sequence used in the synthesis of sub-barcode molecule library
tcgcggatagactcctcgac

SEQ ID NO: 233 - DNA, 20 bp, Artificial Sequence
  Sequence used in the synthesis of sub-barcode molecule library
tcggggatagactcctcgac

SEQ ID NO: 234 - DNA, 20 bp, Artificial Sequence
  Sequence used in the synthesis of sub-barcode molecule library
tcgtggatagactcctcgac

SEQ ID NO: 235 - DNA, 20 bp, Artificial Sequence
  Sequence used in the synthesis of sub-barcode molecule library
tctaggatagactcctcgac

SEQ ID NO: 236 - DNA, 20 bp, Artificial Sequence
  Sequence used in the synthesis of sub-barcode molecule library
tctcggatagactcctcgac

SEQ ID NO: 237 - DNA, 20 bp, Artificial Sequence
  Sequence used in the synthesis of sub-barcode molecule library
tctgggatagactcctcgac

SEQ ID NO: 238 - DNA, 20 bp, Artificial Sequence
  Sequence used in the synthesis of sub-barcode molecule library
tcttggatagactcctcgac

SEQ ID NO: 239 - DNA, 20 bp, Artificial Sequence
  Sequence used in the synthesis of sub-barcode molecule library
tgaaggatagactcctcgac

SEQ ID NO: 240 - DNA, 20 bp, Artificial Sequence
  Sequence used in the synthesis of sub-barcode molecule library
tgacggatagactcctcgac

SEQ ID NO: 241 - DNA, 20 bp, Artificial Sequence
  Sequence used in the synthesis of sub-barcode molecule library
tgagggatagactcctcgac

SEQ ID NO: 242 - DNA, 20 bp, Artificial Sequence
  Sequence used in the synthesis of sub-barcode molecule library
tgatggatagactcctcgac

SEQ ID NO: 243 - DNA, 20 bp, Artificial Sequence
  Sequence used in the synthesis of sub-barcode molecule library
tgcaggatagactcctcgac

SEQ ID NO: 244 - DNA, 20 bp, Artificial Sequence
  Sequence used in the synthesis of sub-barcode molecule library
tgccggatagactcctcgac

SEQ ID NO: 245 - DNA, 20 bp, Artificial Sequence
  Sequence used in the synthesis of sub-barcode molecule library
tgcgggatagactcctcgac

SEQ ID NO: 246 - DNA, 20 bp, Artificial Sequence
  Sequence used in the synthesis of sub-barcode molecule library
tgctggatagactcctcgac

SEQ ID NO: 247 - DNA, 20 bp, Artificial Sequence
  Sequence used in the synthesis of sub-barcode molecule library
tggaggatagactcctcgac

SEQ ID NO: 248 - DNA, 20 bp, Artificial Sequence
  Sequence used in the synthesis of sub-barcode molecule library
tggcggatagactcctcgac

SEQ ID NO: 249 - DNA, 20 bp, Artificial Sequence
  Sequence used in the synthesis of sub-barcode molecule library
tgggggatagactcctcgac

SEQ ID NO: 250 - DNA, 20 bp, Artificial Sequence
  Sequence used in the synthesis of sub-barcode molecule library
tggtggatagactcctcgac

SEQ ID NO: 251 - DNA, 20 bp, Artificial Sequence
  Sequence used in the synthesis of sub-barcode molecule library
tgtaggatagactcctcgac

SEQ ID NO: 252 - DNA, 20 bp, Artificial Sequence
  Sequence used in the synthesis of sub-barcode molecule library
tgtcggatagactcctcgac

SEQ ID NO: 253 - DNA, 20 bp, Artificial Sequence
  Sequence used in the synthesis of sub-barcode molecule library
tgtgggatagactcctcgac

SEQ ID NO: 254 - DNA, 20 bp, Artificial Sequence
  Sequence used in the synthesis of sub-barcode molecule library
tgttggatagactcctcgac

SEQ ID NO: 255 - DNA, 20 bp, Artificial Sequence
  Sequence used in the synthesis of sub-barcode molecule library
ttaaggatagactcctcgac

SEQ ID NO: 256 - DNA, 20 bp, Artificial Sequence
  Sequence used in the synthesis of sub-barcode molecule library
ttacggatagactcctcgac

SEQ ID NO: 257 - DNA, 20 bp, Artificial Sequence
  Sequence used in the synthesis of sub-barcode molecule library
ttagggatagactcctcgac

SEQ ID NO: 258 - DNA, 20 bp, Artificial Sequence
  Sequence used in the synthesis of sub-barcode molecule library
ttatggatagactcctcgac

SEQ ID NO: 259 - DNA, 20 bp, Artificial Sequence
  Sequence used in the synthesis of sub-barcode molecule library
ttcaggatagactcctcgac

SEQ ID NO: 260 - DNA, 20 bp, Artificial Sequence
  Sequence used in the synthesis of sub-barcode molecule library
ttccggatagactcctcgac

SEQ ID NO: 261 - DNA, 20 bp, Artificial Sequence
  Sequence used in the synthesis of sub-barcode molecule library
ttcgggatagactcctcgac

SEQ ID NO: 262 - DNA, 20 bp, Artificial Sequence
  Sequence used in the synthesis of sub-barcode molecule library
ttctggatagactcctcgac

SEQ ID NO: 263 - DNA, 20 bp, Artificial Sequence
  Sequence used in the synthesis of sub-barcode molecule library
ttgaggatagactcctcgac

SEQ ID NO: 264 - DNA, 20 bp, Artificial Sequence
  Sequence used in the synthesis of sub-barcode molecule library
ttgcggatagactcctcgac

SEQ ID NO: 265 - DNA, 20 bp, Artificial Sequence
  Sequence used in the synthesis of sub-barcode molecule library
ttggggatagactcctcgac

SEQ ID NO: 266 - DNA, 20 bp, Artificial Sequence
  Sequence used in the synthesis of sub-barcode molecule library
ttgtggatagactcctcgac

SEQ ID NO: 267 - DNA, 20 bp, Artificial Sequence
  Sequence used in the synthesis of sub-barcode molecule library
tttaggatagactcctcgac

SEQ ID NO: 268 - DNA, 20 bp, Artificial Sequence
  Sequence used in the synthesis of sub-barcode molecule library
tttcggatagactcctcgac

SEQ ID NO: 269 - DNA, 20 bp, Artificial Sequence
  Sequence used in the synthesis of sub-barcode molecule library
tttgggatagactcctcgac

SEQ ID NO: 270 - DNA, 47 bp, Artificial Sequence
  Primer
taatacgactcactatagggagataggacgatacgagtgtgtactcg

SEQ ID NO: 271 - DNA, 31 bp, Artificial Sequence
  Primer
ctgtcaaggtagactagcatgctcccatacg

SEQ ID NO: 272 - DNA, 24 bp, Artificial Sequence
  Primer
ctgtcaaggtagactagcatgctc

SEQ ID NO: 273 - DNA, 60 bp, Artificial Sequence
  Adaptor oligonucleotide
cctgactgctcgtcagttgattaagtactctgtgagatgatgatcagtagagcgagtcgt

SEQ ID NO: 274 - DNA, 50 bp, Artificial Sequence
  Primer
caccgagatctacactctttccctacacgacgctcttccgatcttgacct

SEQ ID NO: 275 - DNA, 59 bp, Artificial Sequence
  Synthetic template
  misc_feature (22)..(39): n is a, c, g, or t
atgatcagtagagcgagtcgtnnnnnnnnnnnnnnnnnntgctacgacttccgagtcca

SEQ ID NO: 276 - DNA, 27 bp, Artificial Sequence
  Primer
gctctactgatcattggactcggaagt

SEQ ID NO: 277 - DNA, 28 bp, Artificial Sequence
  Primer
tccgatcttggactcggaagtcgtagca

SEQ ID NO: 278 - DNA, 39 bp, Artificial Sequence; identical to SEQ ID NO: 17
  Primer

SEQ ID NO: 279 - DNA, 59 bp, Artificial Sequence
  BRCA1 adaptor oligonucleotide
cctgactgctcgtcagttgattaagtactctgtgagatgcttggcccctcttcggtaac

SEQ ID NO: 280 - DNA, 60 bp, Artificial Sequence
  BRCA1 adaptor oligonucleotide
cctgactgctcgtcagttgattaagtactctgtgagatgctgggagctcaaaagatggct

SEQ ID NO: 281 - DNA, 58 bp, Artificial Sequence
  BRCA1 adaptor oligonucleotide
cctgactgctcgtcagttgattaagtactctgtgagatgcagctgggctcaaaggacc

SEQ ID NO: 282 - DNA, 60 bp, Artificial Sequence
  BRCA1 adaptor oligonucleotide
cctgactgctcgtcagttgattaagtactctgtgagatgcagacaaattccccagcaggt

SEQ ID NO: 283 - DNA, 58 bp, Artificial Sequence
  BRCA1 adaptor oligonucleotide
cctgactgctcgtcagttgattaagtactctgtgagatgcatggtgtgaacccgggag

SEQ ID NO: 284 - DNA, 60 bp, Artificial Sequence
  BRCA1 adaptor oligonucleotide
cctgactgctcgtcagttgattaagtactctgtgagatgcccaaatcccaagtcgtgtgt

SEQ ID NO: 285 - DNA, 60 bp, Artificial Sequence
  BRCA1 adaptor oligonucleotide
cctgactgctcgtcagttgattaagtactctgtgagatgctcatccctggttccttgagg

SEQ ID NO: 286 - DNA, 60 bp, Artificial Sequence
  HLA-A adaptor oligonucleotide
cctgactgctcgtcagttgattaagtactctgtgaaaacggcctctgtggggagaagcaa

SEQ ID NO: 287 - DNA, 59 bp, Artificial Sequence
  HLA-A adaptor oligonucleotide
cctgactgctcgtcagttgattaagtactctgtgagatgcactgggctgaccgtggggt

SEQ ID NO: 288 - DNA, 60 bp, Artificial Sequence
  HLA-A adaptor oligonucleotide
cctgactgctcgtcagttgattaagtactctgcctgaatgwtctgactcttcccgtmaga

SEQ ID NO: 289 - DNA, 60 bp, Artificial Sequence
  DQB1 adaptor oligonucleotide
cctgactgctcgtcagttgattaagtactctgggatccccgcagaggatttcgtgtacca

SEQ ID NO: 290 - DNA, 60 bp, Artificial Sequence
  DQB1 adaptor oligonucleotide
cctgactgctcgtcagttgattaagtactctgtgagatggagcccacagtgaccatctcc

SEQ ID NO: 291 - DNA, 60 bp, Artificial Sequence
  BRCA1 reverse primer
cggtctcggcattcctgctgaaccgctcttccgatctgttctgagacacctgatgacctg

SEQ ID NO: 292 - DNA, 57 bp, Artificial Sequence
  BRCA1 reverse primer
cggtctcggcattcctgctgaaccgctcttccgatcttgaacccaggagtttgaggc

SEQ ID NO: 293 - DNA, 60 bp, Artificial Sequence
  BRCA1 reverse primer
cggtctcggcattcctgctgaaccgctcttccgatcttggagctttatctgctctgtgat

SEQ ID NO: 294 - DNA, 57 bp, Artificial Sequence
  BRCA1 reverse primer
cggtctcggcattcctgctgaaccgctcttccgatctttcactgtgatggccaggat

SEQ ID NO: 295 - DNA, 57 bp, Artificial Sequence
  BRCA1 reverse primer
cggtctcggcattcctgctgaaccgctcttccgatcttgacccaagcaagcctaaag

SEQ ID NO: 296 - DNA, 57 bp, Artificial Sequence
  BRCA1 reverse primer
cggtctcggcattcctgctgaaccgctcttccgatcttgccacagtagatgctcagt

SEQ ID NO: 297 - DNA, 58 bp, Artificial Sequence
  BRCA1 reverse primer
cggtctcggcattcctgctgaaccgctcttccgatctcccagcaaccatttcatttca

SEQ ID NO: 298 - DNA, 60 bp, Artificial Sequence
  HLA-A reverse primer
cggtctcggcattcctgctgaaccgctcttccgatcttggatctcggacccggagactgt

SEQ ID NO: 299 - DNA, 58 bp, Artificial Sequence
  HLA-A reverse primer
cggtctcggcattcctgctgaaccgctcttccgatctccctggtaccvgtgcgctgca

SEQ ID NO: 300 - DNA, 60 bp, Artificial Sequence
  HLA-A reverse primer
cggtctcggcattcctgctgaaccgctcttccgatctgaccctgctaaaggtctccagag

SEQ ID NO: 301 - DNA, 57 bp, Artificial Sequence
  HLA-A reverse primer
cggtctcggcattcctgctgaaccgctcttccgatctgaccctgctaaaggtcagag

SEQ ID NO: 302 - DNA, 60 bp, Artificial Sequence
  DQB1 reverse primer
cggtctcggcattcctgctgaaccgctcttccgatctaggacgctcacctctccgctgca

SEQ ID NO: 303 - DNA, 57 bp, Artificial Sequence
  DQB1 reverse primer
cggtctcggcattcctgctgaaccgctcttccgatctctggggtgctccacgtggca

SEQ ID NO: 304 - DNA, 20 bp, Artificial Sequence
  nucleotide sequence
ggcccagcctacacacccat

SEQ ID NO: 305 - DNA, 20 bp, Artificial Sequence
  nucleotide sequence
ttacaagaattatacacctc

SEQ ID NO: 306 - DNA, 20 bp, Artificial Sequence
  nucleotide sequence
ggcccaacctatacgcccat

SEQ ID NO: 307 - DNA, 20 bp, Artificial Sequence
  nucleotide sequence
taacccttgtatttgaacac

SEQ ID NO: 308 - DNA, 20 bp, Artificial Sequence
  nucleotide sequence
ctatccactgattaactgtg

SEQ ID NO: 309 - DNA, 20 bp, Artificial Sequence
  nucleotide sequence
taatcgggccattaagcgat

SEQ ID NO: 310 - DNA, 20 bp, Artificial Sequence
  nucleotide sequence
caagtaatttgctggaccta

SEQ ID NO: 311 - DNA, 16 bp, Artificial Sequence
  nucleotide sequence
taccagagatacttgc

SEQ ID NO: 312 - DNA, 14 bp, Artificial Sequence
  nucleotide sequence
atatccagcaaagt

SEQ ID NO: 313 - DNA, 13 bp, Artificial Sequence
  nucleotide sequence
ttacaagaattat